European Patent Application EP 4 303 301 A1, published January 10, 2024. Title: Prephenate dehydratase variant and method for producing branched amino acid using the same. Applicant: CJ CheilJedang Corporation. The sequence listing filed with the application follows.

SEQUENCE LISTING (47 sequences)

SEQ ID NO: 1 - protein, 315 aa, Artificial Sequence
  PheA_WT
MSDAPTVVAYLGPAGTFTEEALYKFADAGVFGDGEIEQLPAKSPQEAVDAVRHGTAQFAVVAIENFVDGPVTPTFDALDQGSNVQIIAEEELDIAFSIMVRPGTSLADVKTLATHPVGYQQVKNWMATTIPDAMYLSASSNGAGAQMVAEGTADAAAAPSRAAELFGLERLVDDVADVRGARTRFVAVQAQAAVSEPTGHDRTSVIFSLPNVPGSLVRALNEFAIRGVDLTRIESRPTRKVFGTYRFHLDISGHIRDIPVAEALRALHLQAEELVFVGSWPSNRAEDSTPQTDQLAKLHKADEWVRAASEGRKLN

SEQ ID NO: 2 - DNA, 948 bp, Artificial Sequence
  pheA_WT
atgagcgacgcaccaactgttgtggcctatttggggcctgccggaaccttcaccgaagaagccctctacaaatttgccgacgccggcgtattcggcgacggtgagatcgagcagctaccagccaaatcgccacaagaagctgtcgacgccgtccgccacggcaccgcccagttcgcggtggtcgccatcgaaaacttcgtcgacggccccgtcacccccaccttcgacgcccttgaccagggctccaacgtgcaaatcatcgccgaagaagaactcgacatcgccttttccatcatggtccggccagggacttcgcttgccgacgtcaaaaccctcgccacccacccggttgggtaccaacaagtgaaaaactggatggcaaccaccattccggacgccatgtatctttcagcaagctccaacggcgccggcgcacaaatggttgccgaaggaaccgccgacgcagccgcagcgccctcccgcgcagccgaactcttcggactggaacgccttgttgatgatgtcgccgacgtccgtggcgcccgcacccgcttcgttgctgtccaagcccaagcagccgtttccgaaccgaccggccacgaccgcacctccgtcattttctccctaccgaatgtgccaggcagcctcgtgcgcgccctcaacgaattcgccatccgcggcgttgacctcacccgcatcgaatcccgccccacccgcaaagtcttcggaacctaccgcttccacctggacatatccggacatatccgcgatatccccgtcgccgaagccctccgcgcactccacctccaagccgaagaactcgtcttcgtcggctcctggccctccaaccgtgcggaagacagcacgccccaaaccgaccaactagctaagctacacaaggcggacgaatgggttcgcgcagcaagcgaaggaaggaaacttaactag

SEQ ID NO: 3 - DNA, 17 bp, Artificial Sequence
  primer
ttgaggtccttggctgg

SEQ ID NO: 4 - DNA, 18 bp, Artificial Sequence
  primer
cgcaacacgatggagctg

SEQ ID NO: 5 - protein, 315 aa, Artificial Sequence
  PheA_R182A
MSDAPTVVAYLGPAGTFTEEALYKFADAGVFGDGEIEQLPAKSPQEAVDAVRHGTAQFAVVAIENFVDGPVTPTFDALDQGSNVQIIAEEELDIAFSIMVRPGTSLADVKTLATHPVGYQQVKNWMATTIPDAMYLSASSNGAGAQMVAEGTADAAAAPSRAAELFGLERLVDDVADVRGAATRFVAVQAQAAVSEPTGHDRTSVIFSLPNVPGSLVRALNEFAIRGVDLTRIESRPTRKVFGTYRFHLDISGHIRDIPVAEALRALHLQAEELVFVGSWPSNRAEDSTPQTDQLAKLHKADEWVRAASEGRKLN

SEQ ID NO: 6 - DNA, 948 bp, Artificial Sequence
  pheA_R182A
atgagcgacgcaccaactgttgtggcctatttggggcctgccggaaccttcaccgaagaagccctctacaaatttgccgacgccggcgtattcggcgacggtgagatcgagcagctaccagccaaatcgccacaagaagctgtcgacgccgtccgccacggcaccgcccagttcgcggtggtcgccatcgaaaacttcgtcgacggccccgtcacccccaccttcgacgcccttgaccagggctccaacgtgcaaatcatcgccgaagaagaactcgacatcgccttttccatcatggtccggccagggacttcgcttgccgacgtcaaaaccctcgccacccacccggttgggtaccaacaagtgaaaaactggatggcaaccaccattccggacgccatgtatctttcagcaagctccaacggcgccggcgcacaaatggttgccgaaggaaccgccgacgcagccgcagcgccctcccgcgcagccgaactcttcggactggaacgccttgttgatgatgtcgccgacgtccgtggcgccgcgacccgcttcgttgctgtccaagcccaagcagccgtttccgaaccgaccggccacgaccgcacctccgtcattttctccctaccgaatgtgccaggcagcctcgtgcgcgccctcaacgaattcgccatccgcggcgttgacctcacccgcatcgaatcccgccccacccgcaaagtcttcggaacctaccgcttccacctggacatatccggacatatccgcgatatccccgtcgccgaagccctccgcgcactccacctccaagccgaagaactcgtcttcgtcggctcctggccctccaaccgtgcggaagacagcacgccccaaaccgaccaactagctaagctacacaaggcggacgaatgggttcgcgcagcaagcgaaggaaggaaacttaactag

SEQ ID NO: 7 - DNA, 38 bp, Artificial Sequence
  primer
gtgaattcgagctcggtacccgtggcatggatgaaaag

SEQ ID NO: 8 - DNA, 36 bp, Artificial Sequence
  primer
ttggacagcaacgaagcgggtcgcggcgccacggac

SEQ ID NO: 9 - DNA, 37 bp, Artificial Sequence
  primer
gtcgccgacgtccgtggcgccgcgacccgcttcgttg

SEQ ID NO: 10 - DNA, 38 bp, Artificial Sequence
  primer
ggtcgactctagaggatccccgtggctgtccatgattc

SEQ ID NO: 11 - DNA, 21 bp, Artificial Sequence
  primer
tatgcttcaccacatgacttc

SEQ ID NO: 12 - DNA, 23 bp, Artificial Sequence
  primer
aaatcatttgagaaaactcgagg

SEQ ID NO: 13 - DNA, 19 bp, Artificial Sequence
  primer
gtcacccgatcgtctgaag

SEQ ID NO: 14 - DNA, 18 bp, Artificial Sequence
  primer
gtcttaaaaccggttgat

SEQ ID NO: 15 - DNA, 19 bp, Artificial Sequence
  primer
caatgctggctgcgtacgc

SEQ ID NO: 16 - DNA, 20 bp, Artificial Sequence
  primer
ctcctcgcgaggaaccaact

SEQ ID NO: 17 - DNA, 35 bp, Artificial Sequence
  primer
tcgagctcggtaccccgcttttgcactcatcgagc

SEQ ID NO: 18 - DNA, 23 bp, Artificial Sequence
  primer
cacgatcagatgtgcatcatcat

SEQ ID NO: 19 - DNA, 23 bp, Artificial Sequence
  primer
atgatgatgcacatctgatcgtg

SEQ ID NO: 20 - DNA, 35 bp, Artificial Sequence
  primer
ctctagaggatccccgagcatcttccaaaaccttg

SEQ ID NO: 21 - DNA, 35 bp, Artificial Sequence
  primer
tcgagctcggtacccatgagtgaaacatacgtgtc

SEQ ID NO: 22 - DNA, 39 bp, Artificial Sequence
  primer
gcgcttgaggtactctgccagcgcgatgtcatcatccgg

SEQ ID NO: 23 - DNA, 39 bp, Artificial Sequence
  primer
ccggatgatgacatcgcgctggcagagtacctcaagcgc

SEQ ID NO: 24 - DNA, 34 bp, Artificial Sequence
  primer
ctctagaggatcccccgtcaccgacacctccaca

SEQ ID NO: 25 - protein, 437 aa, Artificial Sequence
  GltA_M312I
MFERDIVATDNNKAVLHYPGGEFEMDIIEASEGNNGVVLGKMLSETGLITFDPGYVSTGSTESKITYIDGDAGILRYRGYDIADLAENATFNEVSYLLINGELPTPDELHKFNDEIRHHTLLDEDFKSQFNVFPRDAHPMATLASSVNILSTYYQDQLNPLDEAQLDKATVRLMAKVPMLAAYAHRARKGAPYMYPDNSLNARENFLRMMFGYPTEPYEIDPIMVKALDKLLILHADHEQNCSTSTVRMIGSAQANMFVSIAGGINALSGPLHGGANQAVLEMLEDIKSNHGGDATEFMNKVKNKEDGVRLIGFGHRVYKNYDPRAAIVKETAHEILEHLGGDDLLDLAIKLEEIALADDYFISRKLYPNVDFYTGLIYRAMGFPTDFFTVLFAIGRLPGWIAHYREQLGAAGNKINRPRQVYTGNESRKLVPREER

SEQ ID NO: 26 - DNA, 1314 bp, Artificial Sequence
  gltA_M312I
atgtttgaaagggatatcgtggctactgataacaacaaggctgtcctgcactaccccggtggcgagttcgaaatggacatcatcgaggcttctgagggtaacaacggtgttgtcctgggcaagatgctgtctgagactggactgatcacttttgacccaggttatgtgagcactggctccaccgagtcgaagatcacctacatcgatggcgatgcgggaatcctgcgttaccgcggctatgacatcgctgatctggctgagaatgccaccttcaacgaggtttcttacctacttatcaacggtgagctaccaaccccagatgagcttcacaagtttaacgacgagattcgccaccacacccttctggacgaggacttcaagtcccagttcaacgtgttcccacgcgacgctcacccaatggcaaccttggcttcctcggttaacattttgtctacctactaccaggaccagctgaacccactcgatgaggcacagcttgataaggcaaccgttcgcctcatggcaaaggttccaatgctggctgcgtacgcacaccgcgcacgcaagggtgctccttacatgtacccagacaactccctcaatgcgcgtgagaacttcctgcgcatgatgttcggttacccaaccgagccatacgagatcgacccaatcatggtcaaggctctggacaagctgctcatcctgcacgctgaccacgagcagaactgctccacctccaccgttcgtatgatcggttccgcacaggccaacatgtttgtctccatcgctggtggcatcaacgctctgtccggcccactgcacggtggcgcaaaccaggctgttctggagatgctcgaagacatcaagagcaaccacggtggcgacgcaaccgagttcatgaacaaggtcaagaacaaggaagacggcgtccgcctcatcggcttcggacaccgcgtttacaagaactacgatccacgtgcagcaatcgtcaaggagaccgcacacgagatcctcgagcacctcggtggcgacgatcttctggatctggcaatcaagctggaagaaattgcactggctgatgattacttcatctcccgcaagctctacccgaacgtagacttctacaccggcctgatctaccgcgcaatgggcttcccaactgacttcttcaccgtattgttcgcaatcggtcgtctgccaggatggatcgctcactaccgcgagcagctcggtgcagcaggcaacaagatcaaccgcccacgccaggtctacaccggcaacgaatcccgcaagttggttcctcgcgaggagcgctaa

SEQ ID NO: 27 - DNA, 42 bp, Artificial Sequence
  primer
gtgaattcgagctcggtacccgcgggaatcctgcgttaccgc

SEQ ID NO: 28 - DNA, 42 bp, Artificial Sequence
  primer
tgtaaacgcggtgtccgaagccgatgaggcggacgccgtctt

SEQ ID NO: 29 - DNA, 42 bp, Artificial Sequence
  primer
aagacggcgtccgcctcatcggcttcggacaccgcgtttaca

SEQ ID NO: 30 - DNA, 42 bp, Artificial Sequence
  primer
ggtcgactctagaggatccccttagcgctcctcgcgaggaac

SEQ ID NO: 31 - protein, 436 aa, Artificial Sequence
  IlvA_WT
MSETYVSEKSPGVMASGAELIRAADIQTAQARISSVIAPTPLQYCPRLSEETGAEIYLKREDLQDVRSYKIRGALNSGAQLTQEQRDAGIVAASAGNHAQGVAYVCKSLGVQGRIYVPVQTPKQKRDRIMVHGGEFVSLVVTGNNFDEASAAAHEDAERTGATLIEPFDARNTVIGQGTVAAEILSQLTSMGKSADHVMVPVGGGGLLAGVVSYMADMAPRTAIVGIEPAGAASMQAALHNGGPITLETVDPFVDGAAVKRVGDLNYTIVEKNQGRVHMMSATEGAVCTEMLDLYQNEGIIAEPAGALSIAGLKEMSFAPGSVVVCIISGGNNDVLRYAEIAERSLVHRGLKHYFLVNFPQKPGQLRHFLEDILGPDDDITLFEYLKRNNRETGTALVGIHLSEASGLDSLLERMEESAIDSRRLEPGTPEYEYLT

SEQ ID NO: 32 - DNA, 1311 bp, Artificial Sequence
  ilvA_WT
atgagtgaaacatacgtgtctgagaaaagtccaggagtgatggctagcggagcggagctgattcgtgccgccgacattcaaacggcgcaggcacgaatttcctccgtcattgcaccaactccattgcagtattgccctcgtctttctgaggaaaccggagcggaaatctaccttaagcgtgaggatctgcaggatgttcgttcctacaagatccgcggtgcgctgaactctggagcgcagctcacccaagagcagcgcgatgcaggtatcgttgccgcatctgcaggtaaccatgcccagggcgtggcctatgtgtgcaagtccttgggcgttcagggacgcatctatgttcctgtgcagactccaaagcaaaagcgtgaccgcatcatggttcacggcggagagtttgtctccttggtggtcactggcaataacttcgacgaagcatcggctgcagcgcatgaagatgcagagcgcaccggcgcaacgctgatcgagcctttcgatgctcgcaacaccgtcatcggtcagggcaccgtggctgctgagatcttgtcgcagctgacttccatgggcaagagtgcagatcacgtgatggttccagtcggcggtggcggacttcttgcaggtgtggtcagctacatggctgatatggcacctcgcactgcgatcgttggtatcgaaccagcgggagcagcatccatgcaggctgcattgcacaatggtggaccaatcactttggagactgttgatccctttgtggacggcgcagcagtcaaacgtgtcggagatctcaactacaccatcgtggagaagaaccagggtcgcgtgcacatgatgagcgcgaccgagggcgctgtgtgtactgagatgctcgatctttaccaaaacgaaggcatcatcgcggagcctgctggcgcgctgtctatcgctgggttgaaggaaatgtcctttgcacctggttctgtcgtggtgtgcatcatctctggtggcaacaacgatgtgctgcgttatgcggaaatcgctgagcgctccttggtgcaccgcggtttgaagcactacttcttggtgaacttcccgcaaaagcctggtcagttgcgtcacttcctggaagatatcctgggaccggatgatgacatcacgctgtttgagtacctcaagcgcaacaaccgtgagaccggtactgcgttggtgggtattcacttgagtgaagcatcaggattggattctttgctggaacgtatggaggaatcggcaattgattcccgtcgcctcgagccgggcacccctgagtacgaatacttgacctaa

SEQ ID NO: 33 - DNA, 26 bp, Artificial Sequence
  primer
ggatccgactgagcctgggcaactgg

SEQ ID NO: 34 - DNA, 26 bp, Artificial Sequence
  primer
ggatccccgtcaccgacacctccaca

SEQ ID NO: 35 - DNA, 25 bp, Artificial Sequence
  primer
acatcacgctggcagagtacctcaa

SEQ ID NO: 36 - DNA, 25 bp, Artificial Sequence
  primer
ttgaggtactctgccagcgtgatgt

SEQ ID NO: 37 - protein, 436 aa, Artificial Sequence
  IlvA_T381A, F383A
MSETYVSEKSPGVMASGAELIRAADIQTAQARISSVIAPTPLQYCPRLSEETGAEIYLKREDLQDVRSYKIRGALNSGAQLTQEQRDAGIVAASAGNHAQGVAYVCKSLGVQGRIYVPVQTPKQKRDRIMVHGGEFVSLVVTGNNFDEASAAAHEDAERTGATLIEPFDARNTVIGQGTVAAEILSQLTSMGKSADHVMVPVGGGGLLAGVVSYMADMAPRTAIVGIEPAGAASMQAALHNGGPITLETVDPFVDGAAVKRVGDLNYTIVEKNQGRVHMMSATEGAVCTEMLDLYQNEGIIAEPAGALSIAGLKEMSFAPGSVVVCIISGGNNDVLRYAEIAERSLVHRGLKHYFLVNFPQKPGQLRHFLEDILGPDDDIALAEYLKRNNRETGTALVGIHLSEASGLDSLLERMEESAIDSRRLEPGTPEYEYLT

SEQ ID NO: 38 - DNA, 1311 bp, Artificial Sequence
  ilvA_T381A, F383A
atgagtgaaacatacgtgtctgagaaaagtccaggagtgatggctagcggagcggagctgattcgtgccgccgacattcaaacggcgcaggcacgaatttcctccgtcattgcaccaactccattgcagtattgccctcgtctttctgaggaaaccggagcggaaatctaccttaagcgtgaggatctgcaggatgttcgttcctacaagatccgcggtgcgctgaactctggagcgcagctcacccaagagcagcgcgatgcaggtatcgttgccgcatctgcaggtaaccatgcccagggcgtggcctatgtgtgcaagtccttgggcgttcagggacgcatctatgttcctgtgcagactccaaagcaaaagcgtgaccgcatcatggttcacggcggagagtttgtctccttggtggtcactggcaataacttcgacgaagcatcggctgcagcgcatgaagatgcagagcgcaccggcgcaacgctgatcgagcctttcgatgctcgcaacaccgtcatcggtcagggcaccgtggctgctgagatcttgtcgcagctgacttccatgggcaagagtgcagatcacgtgatggttccagtcggcggtggcggacttcttgcaggtgtggtcagctacatggctgatatggcacctcgcactgcgatcgttggtatcgaaccagcgggagcagcatccatgcaggctgcattgcacaatggtggaccaatcactttggagactgttgatccctttgtggacggcgcagcagtcaaacgtgtcggagatctcaactacaccatcgtggagaagaaccagggtcgcgtgcacatgatgagcgcgaccgagggcgctgtgtgtactgagatgctcgatctttaccaaaacgaaggcatcatcgcggagcctgctggcgcgctgtctatcgctgggttgaaggaaatgtcctttgcacctggttctgtcgtggtgtgcatcatctctggtggcaacaacgatgtgctgcgttatgcggaaatcgctgagcgctccttggtgcaccgcggtttgaagcactacttcttggtgaacttcccgcaaaagcctggtcagttgcgtcacttcctggaagatatcctgggaccggatgatgacatcgcgctggcagagtacctcaagcgcaacaaccgtgagaccggtactgcgttggtgggtattcacttgagtgaagcatcaggattggattctttgctggaacgtatggaggaatcggcaattgattcccgtcgcctcgagccgggcacccctgagtacgaatacttgacctaa

SEQ ID NO: 39 - DNA, 22 bp, Artificial Sequence
  primer
aacacgaccggcatcccgtcgc

SEQ ID NO: 40 - DNA, 23 bp, Artificial Sequence
  primer
aaatcatttgagaaaactcgagg

SEQ ID NO: 41 - DNA, 45 bp, Artificial Sequence
  primer
gtgaattcgagctcggtacccaaatcatttgagaaaactcgaggc

SEQ ID NO: 42 - DNA, 45 bp, Artificial Sequence
  primer
ggtgatcatctcaacggtggaacacaggttgatgatcattgggtt

SEQ ID NO: 43 - DNA, 45 bp, Artificial Sequence
  primer
aacccaatgatcatcaacctgtgttccaccgttgagatgatcacc

SEQ ID NO: 44 - DNA, 42 bp, Artificial Sequence
  primer
ggtcgactctagaggatccccaagaaggcaacatcggacagc

SEQ ID NO: 45 - DNA, 21 bp, Artificial Sequence
  primer
atccattcaatggagtctgcg

SEQ ID NO: 46 - protein, 616 aa, Artificial Sequence
  leuA_P247C, R558H, G561D
MSPNDAFISAPAKIETPVGPRNEGQPAWNKQRGSSMPVNRYMPFEVEVEDISLPDRTWPDKKITVAPQWCAVDLRDGNQALIDPMSPERKRRMFELLVQMGFKEIEVGFPSASQTDFDFVREIIEKGMIPDDVTIQVLVQAREHLIRRTFEACEGAKNVIVHFYNSTSILQRNVVFRMDKVQVKKLATDAAELIKTIAQDYPDTNWRWQYSPESFTGTEVEYAKEVVDAVVEVMDPTPENPMIINLCSTVEMITPNVYADSIEWMHRNLNRRDSIILSLHPHNDRGTGVGAAELGYMAGADRIEGCLFGNGERTGNVCLVTLALNMLTQGVDPQLDFTDIRQIRSTVEYCNQLRVPERHPYGGDLVFTAFSGSHQDAVNKGLDAMAAKVQPGASSTEVSWEQLRDTEWEVPYLPIDPKDVGRDYEAVIRVNSQSGKGGVAYIMKTDHGLQIPRSMQVEFSTVVQNVTDAEGGEVNSKAMWDIFATEYLERTAPVEQIALRVENAQTENEDASITAELIHNGKDVTVDGRGNGPLAAYANALEKLGIDVEIQEYNQHAHTSDDDAEAAAYVLAEVNGRKVWGVGIAGSITYASLKAVTSAVNRALDVNHEAVLAGGV

SEQ ID NO: 47 - DNA, 1851 bp, Artificial Sequence
  leuA_P247C, R558H, G561D
atgtctcctaacgatgcattcatctccgcacctgccaagatcgaaaccccagttgggcctcgcaacgaaggccagccagcatggaataagcagcgtggctcctcaatgccagttaaccgctacatgcctttcgaggttgaggtagaagatatttctctgccggaccgcacttggccagataaaaaaatcaccgttgcacctcagtggtgtgctgttgacctgcgtgacggcaaccaggctctgattgatccgatgtctcctgagcgtaagcgccgcatgtttgagctgctggttcagatgggcttcaaagaaatcgaggtcggtttcccttcagcttcccagactgattttgatttcgttcgtgagatcatcgaaaagggcatgatccctgacgatgtcaccattcaggttctggttcaggctcgtgagcacctgattcgccgtacttttgaagcttgcgaaggcgcaaaaaacgttatcgtgcacttctacaactccacctccatcctgcagcgcaacgtggtgttccgcatggacaaggtgcaggtgaagaagctggctaccgatgccgctgaactaatcaagaccatcgctcaggattacccagacaccaactggcgctggcagtactcccctgagtccttcaccggcactgaggttgagtacgccaaggaagttgtggacgcagttgttgaggtcatggatccaactcctgagaacccaatgatcatcaacctgtgttccaccgttgagatgatcacccctaacgtttacgcagactccattgaatggatgcaccgcaatctaaaccgtcgtgattccattatcctgtccctgcacccgcacaatgaccgtggcaccggcgttggcgcagctgagctgggctacatggctggcgctgaccgcatcgaaggctgcctgttcggcaacggcgagcgcaccggcaacgtctgcctggtcaccctggcactgaacatgctgacccagggcgttgaccctcagctggacttcaccgatatacgccagatccgcagcaccgttgaatactgcaaccagctgcgcgttcctgagcgccacccatacggcggtgacctggtcttcaccgctttctccggttcccaccaggacgctgtgaacaagggtctggacgccatggctgccaaggttcagccaggtgctagctccactgaagtttcttgggagcagctgcgcgacaccgaatgggaggttccttacctgcctatcgatccaaaggatgtcggtcgcgactacgaggctgttatccgcgtgaactcccagtccggcaagggcggcgttgcttacatcatgaagaccgatcacggtctgcagatccctcgctccatgcaggttgagttctccaccgttgtccagaacgtcaccgacgctgagggcggcgaggtcaactccaaggcaatgtgggatatcttcgccaccgagtacctggagcgcaccgcaccagttgagcagatcgcgctgcgcgtcgagaacgctcagaccgaaaacgaggatgcatccatcaccgccgagctcatccacaacggcaaggacgtcaccgtcgatggccgcggcaacggcccactggccgcttacgccaacgcgctggagaagctgggcatcgacgttgagatccaggaatacaaccagcacgcccacacctcggatgacgatgcagaagcagccgcctacgtgctggctgaggtcaacggccgcaaggtctggggcgtcggcatcgctggctccatcacctacgcttcgctgaaggcagtgacctccgccgtaaaccgcgcgctggacgtcaaccacgaggcagtcctggctggcggcgtttaa